European Patent Specification EP 3 808 775 B1, published April 17, 2024. Title: NON-HUMAN ANIMALS HAVING A HUMANIZED CLUSTER OF DIFFERENTIATION 274 GENE. Applicant: REGENERON PHARMACEUTICALS, INC. Application EP. The sequence listing filed with the application follows.

SEQUENCE LISTING (38 sequences)

SEQ ID NO: 1 - DNA, 3653 bp, Mus musculus
gaaatcgtggtccccaagcctcatgccaggctgcacttgcacgtcgcgggccagtctcctcgcctgcagatagttcccaaaacatgaggatatttgctggcattatattcacagcctgctgtcacttgctacgggcgtttactatcacggctccaaaggacttgtacgtggtggagtatggcagcaacgtcacgatggagtgcagattccctgtagaacgggagctggacctgcttgcgttagtggtgtactgggaaaaggaagatgagcaagtgattcagtttgtggcaggagaggaggaccttaagcctcagcacagcaacttcagggggagagcctcgctgccaaaggaccagcttttgaagggaaatgctgcccttcagatcacagacgtcaagctgcaggacgcaggcgtttactgctgcataatcagctacggtggtgcggactacaagcgaatcacgctgaaagtcaatgccccataccgcaaaatcaaccagagaatttccgtggatccagccacttctgagcatgaactaatatgtcaggccgagggttatccagaagctgaggtaatctggacaaacagtgaccaccaacccgtgagtgggaagagaagtgtcaccacttcccggacagaggggatgcttctcaatgtgaccagcagtctgagggtcaacgccacagcgaatgatgttttctactgtacgttttggagatcacagccagggcaaaaccacacagcggagctgatcatcccagaactgcctgcaacacatcctccacagaacaggactcactgggtgcttctgggatccatcctgttgttcctcattgtagtgtccacggtcctcctcttcttgagaaaacaagtgagaatgctagatgtggagaaatgtggcgttgaagatacaagctcaaaaaaccgaaatgatacacaattcgaggagacgtaagcagtgttgaaccctctgatcgtcgattggcagcttgtggtctgtgaaagaaagggcccatgggacatgagtccaaagactcaagatggaacctgagggagagaaccaagaaagtgttgggagaggagcctggaacaacggacattttttccagggagacactgctaagcaagttgcccatcagtcgtcttgggaaatggattgagggttcctggcttagcagctggtccttgcacagtgaccttttcctctgctcagtgccgggatgagagatggagtcatgagtgttgaagaataagtgccttctatttattttgagtctgtgtgttctcactttgggcatgtaattatgactggtgaattctgacgacatgatagatcttaagatgtagtcaccaaactcaactgctgcttagcatcctccgtaactactgatacaagcagggaacacagaggtcacctgcttggtttgacaggctcttgctgtctgactcaaataatctttatttttcagtcctcaaggctcttcgatagcagttgttctgtatcagccttataggtgtcaggtatagcactcaacatctcatctcattacaatagcaaccctcatcaccatagcaacagctaacctctgttatcctcacttcatagccaggaagctgagcgactaagtcacttgcccacagagtatcagctctcagatttctgttcttcagccactgtcctttcaggatagaatttgtcgttaagaaattaatttaaaaactgattattgagtagcattgtatatcaatcacaacatgccttgtgcactgtgctggcctctgagcataaagatgtacgccggagtaccggtcggacatgtttatgtgtgttaaatactcagagaaatgttcattaacaaggagcttgcattttagagacactggaaagtaactccagttcattgtctagcattacatttacctcatttgctatccttgccatacagtctcttgttctccatgaagtgtcatgaatcttgttgaatagttcttttattttttaaatgtttctatttaaatgatattgacatctgaggcgatagctcagttggtaaaaccctttcctcacaagtgtgaaaccctgagtcttatccctagaacccacataaaaaacagttgcgtatgtttgtgcatgcttttgatcccagcactagggaggcagaggcaggcagatcctgagctctcattgaccacccagcctagcctacatggttagctccaggcctacaggagctggcagagcctgaaaaacgatgcctagacacacacacacacacacacacacacacacacacacacacacaccatgtactcatagacctaagtgcaccctcctacacatgcacacacatacaattcaaacacaaatcaacagggaattgtctcagaatggtccccaagacaaagaagaagaaaaacaccaaaccagctctattccctcagcctatcctctctactccttcctagaagcaactactattgtttttgtatataaatttacccaacgacagttaatatgtagaatatatattaaagtgtctgtcaatatatattatctctttctttctttcttcctttctttctttctttctttctttctttctttctttctttctttctttcttccttccttccttccttccttccttccttccttcctttctttctttctttctttttttctgtctatctgtacctaaatggttgctcactatgcattttctgtgctcttcgccctttttatttaatgtatggatatttatgctgcttccagaatggatctaaagctctttgtttctaggttttctcccccatccttctaggcatctctcacactgtctaggccagacaccatgtctgctgcctgaatctgtagacaccatttataaagcacgtactcaccgagtttgtatttggcttgttctgtgtctgattaaagggagaccatgagtccccagggtacactgagttaccccagtaccaagggggagccttgtttgtgtctccatggcagaagcaggcctggagccattttggtttcttccttgacttctctcaaacacagacgcctcacttgctcattacaggttctcctttgggaatgtcagcattgctccttgactgctggctgccctggaaggagcccattagctctgtgtgagcccttgacagctactgcctctccttaccacaggggcctctaagatactgttacctagaggtcttgaggatctgtgttctctggggggaggaaaggaggaggaacccagaactttcttacagttttccttgttctgtcacatgtcaagactgaaggaacaggctgggctacgtagtgagatcctgtctcaaaggaaagacgagcatagccgaacccccggtggaaccccctctgttacctgttcacacaagcttattgatgagtctcatgttaatgtcttgtttgtatgaagtttaagaaaatatcgggttgggcaacacattctatttattcattttatttgaaatcttaatgccatctcatggtgttggattggtgtggcactttattcttttgtgttgtgtataaccataaattttattttgcatcagattgtcaatgtattgcattaatttaataaatatttttatttattaaaaaaaaaaaaaaaaa

SEQ ID NO: 2 - protein, 290 aa, Mus musculus
MRIFAGIIFTACCHLLRAFTITAPKDLYVVEYGSNVTMECRFPVERELDLLALVVYWEKEDEQVIQFVAGEEDLKPQHSNFRGRASLPKDQLLKGNAALQITDVKLQDAGVYCCIISYGGADYKRITLKVNAPYRKINQRISVDPATSEHELICQAEGYPEAEVIWTNSDHQPVSGKRSVTTSRTEGMLLNVTSSLRVNATANDVFYCTFWRSQPGQNHTAELIIPELPATHPPQNRTHWVLLGSILLFLIVVSTVLLFLRKQVRMLDVEKCGVEDTSSKNRNDTQFEET

SEQ ID NO: 3 - DNA, 3691 bp, Homo sapiens
ggcgcaacgctgagcagctggcgcgtcccgcgcggccccagttctgcgcagcttcccgaggctccgcaccagccgcgcttctgtccgcctgcagggcattccagaaagatgaggatatttgctgtctttatattcatgacctactggcatttgctgaacgcatttactgtcacggttcccaaggacctatatgtggtagagtatggtagcaatatgacaattgaatgcaaattcccagtagaaaaacaattagacctggctgcactaattgtctattgggaaatggaggataagaacattattcaatttgtgcatggagaggaagacctgaaggttcagcatagtagctacagacagagggcccggctgttgaaggaccagctctccctgggaaatgctgcacttcagatcacagatgtgaaattgcaggatgcaggggtgtaccgctgcatgatcagctatggtggtgccgactacaagcgaattactgtgaaagtcaatgccccatacaacaaaatcaaccaaagaattttggttgtggatccagtcacctctgaacatgaactgacatgtcaggctgagggctaccccaaggccgaagtcatctggacaagcagtgaccatcaagtcctgagtggtaagaccaccaccaccaattccaagagagaggagaagcttttcaatgtgaccagcacactgagaatcaacacaacaactaatgagattttctactgcacttttaggagattagatcctgaggaaaaccatacagctgaattggtcatcccagaactacctctggcacatcctccaaatgaaaggactcacttggtaattctgggagccatcttattatgccttggtgtagcactgacattcatcttccgtttaagaaaagggagaatgatggatgtgaaaaaatgtggcatccaagatacaaactcaaagaagcaaagtgatacacatttggaggagacgtaatccagcattggaacttctgatcttcaagcagggattctcaacctgtggtttaggggttcatcggggctgagcgtgacaagaggaaggaatgggcccgtgggatgcaggcaatgtgggacttaaaaggcccaagcactgaaaatggaacctggcgaaagcagaggaggagaatgaagaaagatggagtcaaacagggagcctggagggagaccttgatactttcaaatgcctgaggggctcatcgacgcctgtgacagggagaaaggatacttctgaacaaggagcctccaagcaaatcatccattgctcatcctaggaagacgggttgagaatccctaatttgagggtcagttcctgcagaagtgccctttgcctccactcaatgcctcaatttgttttctgcatgactgagagtctcagtgttggaacgggacagtatttatgtatgagtttttcctatttattttgagtctgtgaggtcttcttgtcatgtgagtgtggttgtgaatgatttcttttgaagatatattgtagtagatgttacaattttgtcgccaaactaaacttgctgcttaatgatttgctcacatctagtaaaacatggagtatttgtaaggtgcttggtctcctctataactacaagtatacattggaagcataaagatcaaaccgttggttgcataggatgtcacctttatttaacccattaatactctggttgacctaatcttattctcagacctcaagtgtctgtgcagtatctgttccatttaaatatcagctttacaattatgtggtagcctacacacataatctcatttcatcgctgtaaccaccctgttgtgataaccactattattttacccatcgtacagctgaggaagcaaacagattaagtaacttgcccaaaccagtaaatagcagacctcagactgccacccactgtccttttataatacaatttacagctatattttactttaagcaattcttttattcaaaaaccatttattaagtgcccttgcaatatcaatcgctgtgccaggcattgaatctacagatgtgagcaagacaaagtacctgtcctcaaggagctcatagtataatgaggagattaacaagaaaatgtattattacaatttagtccagtgtcatagcataaggatgatgcgaggggaaaacccgagcagtgttgccaagaggaggaaataggccaatgtggtctgggacggttggatatacttaaacatcttaataatcagagtaattttcatttacaaagagaggtcggtacttaaaataaccctgaaaaataacactggaattccttttctagcattatatttattcctgatttgcctttgccatataatctaatgcttgtttatatagtgtctggtattgtttaacagttctgtcttttctatttaaatgccactaaattttaaattcatacctttccatgattcaaaattcaaaagatcccatgggagatggttggaaaatctccacttcatcctccaagccattcaagtttcctttccagaagcaactgctactgcctttcattcatatgttcttctaaagatagtctacatttggaaatgtatgttaaaagcacgtatttttaaaatttttttcctaaatagtaacacattgtatgtctgctgtgtactttgctatttttatttattttagtgtttcttatatagcagatggaatgaatttgaagttcccagggctgaggatccatgccttctttgtttctaagttatctttcccatagcttttcattatctttcatatgatccagtatatgttaaatatgtcctacatatacatttagacaaccaccatttgttaagtatttgctctaggacagagtttggatttgtttatgtttgctcaaaaggagacccatgggctctccagggtgcactgagtcaatctagtcctaaaaagcaatcttattattaactctgtatgacagaatcatgtctggaacttttgttttctgctttctgtcaagtataaacttcactttgatgctgtacttgcaaaatcacattttctttctggaaattccggcagtgtaccttgactgctagctaccctgtgccagaaaagcctcattcgttgtgcttgaacccttgaatgccaccagctgtcatcactacacagccctcctaagaggcttcctggaggtttcgagattcagatgccctgggagatcccagagtttcctttccctcttggccatattctggtgtcaatgacaaggagtaccttggctttgccacatgtcaaggctgaagaaacagtgtctccaacagagctccttgtgttatctgtttgtacatgtgcatttgtacagtaattggtgtgacagtgttctttgtgtgaattacaggcaagaattgtggctgagcaaggcacatagtctactcagtctattcctaagtcctaactcctccttgtggtgttggatttgtaaggcactttatcccttttgtctcatgtttcatcgtaaatggcataggcagagatgatacctaattctgcatttgattgtcactttttgtacctgcattaatttaataaaatattcttatttattttgttacttggtacaccagcatgtccattttcttgtttattttgtgtttaataaaatgttcagtttaacatcccagtggagaaagttaaaaaa

SEQ ID NO: 4 - protein, 290 aa, Homo sapiens
MRIFAVFIFMTYWHLLNAFTVTVPKDLYVVEYGSNMTIECKFPVEKQLDLAALIVYWEMEDKNIIQFVHGEEDLKVQHSSYRQRARLLKDQLSLGNAALQITDVKLQDAGVYRCMISYGGADYKRITVKVNAPYNKINQRILVVDPVTSEHELTCQAEGYPKAEVIWTSSDHQVLSGKTTTTNSKREEKLFNVTSTLRINTTTNEIFYCTFRRLDPEENHTAELVIPELPLAHPPNERTHLVILGAILLCLGVALTFIFRLRKGRMMDVKKCGIQDTNSKKQSDTHLEET

SEQ ID NO: 5 - DNA, 3656 bp, Artificial Sequence
  Polynucleotide (humanized CD274 mRNA)
gaaatcgtggtccccaagcctcatgccaggctgcacttgcacgtcgcgggccagtctcctcgcctgcagatagttcccaaaacatgaggatatttgctggcattatattcacagcctgctgtcacttgctacgggcatttactgtcacggttcccaaggacctatatgtggtagagtatggtagcaatatgacaattgaatgcaaattcccagtagaaaaacaattagacctggctgcactaattgtctattgggaaatggaggataagaacattattcaatttgtgcatggagaggaagacctgaaggttcagcatagtagctacagacagagggcccggctgttgaaggaccagctctccctgggaaatgctgcacttcagatcacagatgtgaaattgcaggatgcaggggtgtaccgctgcatgatcagctatggtggtgccgactacaagcgaattactgtgaaagtcaatgccccatacaacaaaatcaaccaaagaattttggttgtggatccagtcacctctgaacatgaactgacatgtcaggctgagggctaccccaaggccgaagtcatctggacaagcagtgaccatcaagtcctgagtggtaagaccaccaccaccaattccaagagagaggagaagcttttcaatgtgaccagcacactgagaatcaacacaacaactaatgagattttctactgcacttttaggagattagatcctgaggaaaaccatacagctgaattggtcatcccagaactacctctggcacatcctccaaatgaaaggactcactgggtgcttctgggatccatcctgttgttcctcattgtagtgtccacggtcctcctcttcttgagaaaacaagtgagaatgctagatgtggagaaatgtggcgttgaagatacaagctcaaaaaaccgaaatgatacacaattcgaggagacgtaagcagtgttgaaccctctgatcgtcgattggcagcttgtggtctgtgaaagaaagggcccatgggacatgagtccaaagactcaagatggaacctgagggagagaaccaagaaagtgttgggagaggagcctggaacaacggacattttttccagggagacactgctaagcaagttgcccatcagtcgtcttgggaaatggattgagggttcctggcttagcagctggtccttgcacagtgaccttttcctctgctcagtgccgggatgagagatggagtcatgagtgttgaagaataagtgccttctatttattttgagtctgtgtgttctcactttgggcatgtaattatgactggtgaattctgacgacatgatagatcttaagatgtagtcaccaaactcaactgctgcttagcatcctccgtaactactgatacaagcagggaacacagaggtcacctgcttggtttgacaggctcttgctgtctgactcaaataatctttatttttcagtcctcaaggctcttcgatagcagttgttctgtatcagccttataggtgtcaggtatagcactcaacatctcatctcattacaatagcaaccctcatcaccatagcaacagctaacctctgttatcctcacttcatagccaggaagctgagcgactaagtcacttgcccacagagtatcagctctcagatttctgttcttcagccactgtcctttcaggatagaatttgtcgttaagaaattaatttaaaaactgattattgagtagcattgtatatcaatcacaacatgccttgtgcactgtgctggcctctgagcataaagatgtacgccggagtaccggtcggacatgtttatgtgtgttaaatactcagagaaatgttcattaacaaggagcttgcattttagagacactggaaagtaactccagttcattgtctagcattacatttacctcatttgctatccttgccatacagtctcttgttctccatgaagtgtcatgaatcttgttgaatagttcttttattttttaaatgtttctatttaaatgatattgacatctgaggcgatagctcagttggtaaaaccctttcctcacaagtgtgaaaccctgagtcttatccctagaacccacataaaaaacagttgcgtatgtttgtgcatgcttttgatcccagcactagggaggcagaggcaggcagatcctgagctctcattgaccacccagcctagcctacatggttagctccaggcctacaggagctggcagagcctgaaaaacgatgcctagacacacacacacacacacacacacacacacacacacacacacaccatgtactcatagacctaagtgcaccctcctacacatgcacacacatacaattcaaacacaaatcaacagggaattgtctcagaatggtccccaagacaaagaagaagaaaaacaccaaaccagctctattccctcagcctatcctctctactccttcctagaagcaactactattgtttttgtatataaatttacccaacgacagttaatatgtagaatatatattaaagtgtctgtcaatatatattatctctttctttctttcttcctttctttctttctttctttctttctttctttctttctttctttctttcttccttccttccttccttccttccttccttccttcctttctttctttctttctttttttctgtctatctgtacctaaatggttgctcactatgcattttctgtgctcttcgccctttttatttaatgtatggatatttatgctgcttccagaatggatctaaagctctttgtttctaggttttctcccccatccttctaggcatctctcacactgtctaggccagacaccatgtctgctgcctgaatctgtagacaccatttataaagcacgtactcaccgagtttgtatttggcttgttctgtgtctgattaaagggagaccatgagtccccagggtacactgagttaccccagtaccaagggggagccttgtttgtgtctccatggcagaagcaggcctggagccattttggtttcttccttgacttctctcaaacacagacgcctcacttgctcattacaggttctcctttgggaatgtcagcattgctccttgactgctggctgccctggaaggagcccattagctctgtgtgagcccttgacagctactgcctctccttaccacaggggcctctaagatactgttacctagaggtcttgaggatctgtgttctctggggggaggaaaggaggaggaacccagaactttcttacagttttccttgttctgtcacatgtcaagactgaaggaacaggctgggctacgtagtgagatcctgtctcaaaggaaagacgagcatagccgaacccccggtggaaccccctctgttacctgttcacacaagcttattgatgagtctcatgttaatgtcttgtttgtatgaagtttaagaaaatatcgggttgggcaacacattctatttattcattttatttgaaatcttaatgccatctcatggtgttggattggtgtggcactttattcttttgtgttgtgtataaccataaattttattttgcatcagattgtcaatgtattgcattaatttaataaatatttttatttattaaaaaaaaaaaaaaaaa

SEQ ID NO: 6 - protein, 291 aa, Artificial Sequence
  Polypeptide (humanized CD274 amino acid)
MRIFAGIIFTACCHLLRAFTVTVPKDLYVVEYGSNMTIECKFPVEKQLDLAALIVYWEMEDKNIIQFVHGEEDLKVQHSSYRQRARLLKDQLSLGNAALQITDVKLQDAGVYRCMISYGGADYKRITVKVNAPYNKINQRILVVDPVTSEHELTCQAEGYPKAEVIWTSSDHQVLSGKTTTTNSKREEKLFNVTSTLRINTTTNEIFYCTFRRLDPEENHTAELVIPELPLAHPPNERTHWVLLGSILLFLIVVSTVLLFLRKQVRMLDVEKCGVEDTSSKNRNDTQFEET

SEQ ID NO: 7 - DNA, 13440 bp, Artificial Sequence
  Polynucleotide (humanization fragment A)
gtcacggttcccaaggacctatatgtggtagagtatggtagcaatatgacaattgaatgcaaattcccagtagaaaaacaattagacctggctgcactaattgtctattgggaaatggaggataagaacattattcaatttgtgcatggagaggaagacctgaaggttcagcatagtagctacagacagagggcccggctgttgaaggaccagctctccctgggaaatgctgcacttcagatcacagatgtgaaattgcaggatgcaggggtgtaccgctgcatgatcagctatggtggtgccgactacaagcgaattactgtgaaagtcaatggtaagaattattatagatgagaggcctgatctttattgaaaacatattccaagtgttgaagacttttcattcttgtaagtccatacttattttcaaacagaacagcatagtctgttcattcattcattcaattcatgaattcattcacataattatccaatttcttgagcacctatttgatagtcactggaaatccagagacaaacaacacagagccatgttctacagtatgtacagttttccaaaaagaatttctagtctttacttttttattacaaatggaatacgtatacttgcaaataattcagatactgtggaagagatcaaatgaattgcaaaagtgtccctcctcccttcaccactatctcccatggcatgcagagagagtaaccattatttgtgtgtccctccagaaatttttttattcaactactatttttttattttattaggtccgtcagttttccttttttgagcctctctatatcaaatgcaaataaatatattcagaacaaaccccactgtaaggttcacattaaaaaagacttgaagtcaccctatgaagacaaaaaataatcacattaagtgtgaaagaacctattcttccagtacaggataagccatacttactgggcatatattcatcttgaaaatctatactgatgttgtcttggggaattgaaaaggaactaggagtgttagttcctcggtattgacccacagttatgttatcaggtcacttgagttcaaagttttgtgttggcactagctaagtaaaggaaaacacctctgctttcattgttgagtttcacagaattgagagctgaaaggatcccaggcaggagcagctaatccaaactcccacaaagaacaaaaatcccccagaggatcttctgttcttatatttcctgcaatggcgtccctgtcatatcccacaatggcctccctgccatttggatatcccttccatatcctgttgaaattactccctaatagtaagctgaaatctgcccctctagttgtagtcttgggattatttcatttacatgatgaccttttaatatttgactagaattaaatcatctccccttggtctttccattcctgggctaactaccatcaatctgagggctaacaatacaagtagaaaaagtatacatttgtcactgatcactgatcaattattaatcaatgatcactgataactataaactcaaaaacaaaatcatgtggggattaagagaaatgtatcagttttatgttgtatttctggtccctgatactggctcaggtaatgccactattgtcaagaagataccacttgtaaagtagatttaattttcattatattttaccatatgcttctccattcatgacatctcttgagatgttgtggtttatactttcagtttttctccagtccatccgcaaatatcaggcatctactgtgttccaagatattaaagaaatcatcatgacttagcctcatcaacagcattgctagatctgggatggaaaggaagagtataatcctggcagtcaggaagaaggcagcataaagtataagtttctgcttccaaaaaaggtctctcatcagcctgtagggagtgtgtagggaagggacagctgtccttgtagtagggaagggttttattcaggtcgtctgggctccataatatcccttgtgtatctgcagtctcctttgccatggatcaacacaataggaaatcttccggcactgatggtttttccaagggggagttcttcctggagcaaagcaaatgaccaaccaggtttgaggacctgatttgtttgacaattccattttgtattgtaaattacttaattggcattctactcccaatccatcttgtcatttgcatacagtggttttgggattgagttcagctataccaaaagtctgaaccttctgcacttagaacaaggcaaccaccaagcttcacttgcactgaggccgtgtctccaatggaaatgaggcagctggcttgcaggagcttcccaactcagggaagtagaactcctgagtcacctccatatgcaaatgatttcacagtaatgctgttgaacttcacttcccatcacagcaaatgtgtggtaacatagcttccccacaggagtttactcaccatggtattttaaaggtgaaacatttcaaaactgaaatttgaaagaatttagttttggattcactcaattatcactatcacttcgggtgttattgcacctttcttgtttgtgagtttaaatgccagactctcaggccactaactttcaattaaaagtgtttttctttaatcgctgaacctaacagcagggaaaacgaaatgttcattcagactttcagaaccttcaatgagattaggcagctgaaagatcaaagtgttgcatagttgtcccgataaagctatttggatcatatggaccaaatcgactgctgtcattccccaccaaccccatctctccccaaaattcccagccctgtttaagtgttctctgtagcatttatctctatctagtatattgtgtagcatatcatatcatacttttctgttttgtttattgtctctctcctcctagaatataaactccacaagcacaaagatttgggcctgttttataatattgttgcatccccagggcctgatatacagcagagtggtggtacgaaaagagcacacaaaaaaatatttgttgagtcaatgaatgaatgatttcctcaaataggattagcctaaaattttggaaacatgaacagatttggatatgtgaaaatttatttccagactgttcatcaggaactgttagcagcttctaaagggtacactggagcagcagtagtaaaaggaggaagaggagcagctctgctactgctactatcgagtactactacaattagcacttgcttattctgtgtgttaggccctgtactgaacactctgtctaaattagttcatttcctcctggaaatgactctagggggtaagtgcttcatcatgtaagatgagtatttttcacattttgttgtgtctgaaatctgagtgtgtctttcaatgatggaatctttgattccatgataagtggtattattcccattttaaggatgaggaaactgaggtccaaagaaattaagtaatttgcccaaattcacccagcctagaaaatgataaagctagttctaaacccaagcagattagctctgaagtctgggcccttaataaccactttttattgcctatatttgtacctctggtgtacgtatcaagttatatgttgacttcaaaactatcatgaccttttcttggttttgattgtccaacattagtatagtgttctgggtctgcaaaaattttgattactcatctcatctgtaaaacattttgaactcgtgtgtttgtgcatgcacatttgtgtgtaattataaaaattttactttctgttaatatataagttgtatcataagaaactgccgtttttgaagagcaaaaaaaggttgaatgttaccagttacatctggttcaacctaatagacatttgtacaaaaacagacattttaagaggttgaaataaaaatttaataaacaatattttcagtttttactaattgtgatgcttcactatcattagctaatatgtcaaggcataatataccttagggtgaactttatcattaacaaaggtggatggtgtcaataatcttgaggtttgtgtttttttatataacactgcgaggtctaattaagtacttactgtttaccacctcatacagtggccgataaaaagtgtcacttctgctgtttcctctgggttgtgcttgaattattagtattatcttcagtcctcagtttctttgtgggaaactttttaattagttgtttaattttgtaagatggttagtttagtcaaaattagataagagaatttgaaaatccgtagctaccccaaagcaacctacacataagaactattatttttgtgttttgaaatcataattttattgatttccagtgtttccactggtagtggtttcattgatataggagtatcaaaacatcactcattatttatttcagtttcatttgatcctagccgttttgtattaactctctgtgaagaaattacctcacaaatctattgctgtcgctagctcgctaccttaggaccgttatagttactagcataacttcgtatagcatacattatacgaagttattccagacatgataagatacattgatgagtttggacaaaccacaactagaatgcagtgaaaaaaatgctttatttgtgaaatttgtgatgctattgctttatttgtaaccattataagctgcaataaacaagttaacaacaacaattgcattcattttatgtttcaggttcagggggaggtgtgggaggttttttaaagcaagtaaaacctctacagatgtgatatggctgattatgatcattacttatctagagcttagatcccccctgcccggttattattatttttgacaccagaccaactggtaatggtgcggaggcacgctcagctggaattggccgcaactagggcaggtttaacaacaacaattgcattcattttatgtttcaggttcagggggaggtgtgggaggttttttaaagcaagtaaaacctctacagatgtgatatggctgattatgatcattacttatctagatcaatcgccatcttccagcaggcgcaccattgcccctgtttcactatccaggttacggatatagttcatgacaatatttacattggtccagccaccagcttgcatgatctccggtattgaaactccagcgcgggccatatctcgcgcggctccgacacgggcactgtgtccagaccaggccaggtatctctgaccagagtcatcctaaaatacacaaacaattagaatcagtagtttaacacattatacacttaaaaattttatatttaccttagcgccgtaaatcaatcgatgagttgcttcaaaaatcccttccagggcgcgagttgatagctggctggtggcagatggcgcggcaacaccattttttctgacccggcaaaacaggtagttattcggatcatcagctacaccagagacggaaatccatcgctcgaccagtttagttacccccaggctaagtgccttctctacacctgcggtgctaaccagcgttttcgttctgccaatatggattaacattctcccaccgtcagtacgtgagatatctttaaccctgatcctggcaatttcggctatacgtaacagggtgttataagcaatccccagaaatgccagattacgtatatcctggcagcgatcactattttccatgagtgaacgaacctggtcgaaatcagtgcgttcgaacgctagagcctgttttgcacgttcaccggcatcaacgttttcttttcggatccgccgcataaccagtgaaacagcattgctgtcacttggtcgtggcagcccggaccgacgatgaagcatgtttagctggcccaaatgttgctggatagtttttactgccagaccgcgcgcctgaagatatagaagataatcgcgaacatcttcaggttctgcgggaaaccatttccggttattcaacttgcaccatgccgcccacgaccggcaaacggacagaagcattttccaggtatgctcagaaaacgcctggcgatccctgaacatgtccatcaggttcttgcgaacctcatcactcgttgcatcgaccggtaatgcaggcaaattttggtgtacggtcagtaaattggaatttaaatcggtacgcaccttcctcttcttcttgggggtacccatggtgctggcttggccgggagctggctcagagcaggggacaccacctgggtcgagccagccaacctgtgagcaggtggaattttgtgggctgtggcctgggagccagcaccctcttcctcttatagatactagtggcccctaggaattatgaagtcaaagaggaccaggacctcacagaccatggccagtgaggacctgtaccatgtccaaatatgggcatgagaggggtgggcagggctttggcatcaggagttgcttgtgtcacagtcaagaagtgacaaagatggcatccacttgagtgttcagttagtcactcagcttaggtgttaagtgccacacacctgcttctaggctaggtcctgatagataacccaaggccaggcaggtgggtgaaacagccacatggatttgaactgtgaaaagcacacatcttcagactgctcagagaatgctgctgagggaacttgaccttttaagaaattatccaacgccccagtgaggcactgacagacaaatccagagggtctcagagttgcaggggggtgggctctagtaaaacattgaggccccatcaagtgcttcaggtataaatgggagccacatggatgcagagcagtgtttggactgagggaggtgttggacattactagacagaaggtggacgtgggtgctgctactggcgcccgggctaggggctgcaggtcgaggtctgatggaattagaacttggcaaaacaatactgagaatgaagtgtatgtggaacagaggctgctgatctcgttcttcaggctatgaaactgacacatttggaaaccacagtacttagaaccacaaagtgggaatcaagagaaaaacaatgatcccacgagagatctatagatctatagatcatgagtgggaggaatgagctggcccttaatttggttttgcttgtttaaattatgatatccaactatgaaacattatcataaagcaatagtaaagagccttcagtaaagagcaggcatttatctaatcccaccccacccccacccccgtagctccaatccttccattcaaaatgtaggtactctgttctcacccttcttaacaaagtatgacaggaaaaacttccattttagtggacatctttattgtttaatagatcatcaatttctgcagacttacagcggatcccctcagaagaactcgtcaagaaggcgatagaaggcgatgcgctgcgaatcgggagcggcgataccgtaaagcacgaggaagcggtcagcccattcgccgccaagctcttcagcaatatcacgggtagccaacgctatgtcctgatagcggtccgccacacccagccggccacagtcgatgaatccagaaaagcggccattttccaccatgatattcggcaagcaggcatcgccatgggtcacgacgagatcatcgccgtcgggcatgcgcgccttgagcctggcgaacagttcggctggcgcgagcccctgatgctcttcgtccagatcatcctgatcgacaagaccggcttccatccgagtacgtgctcgctcgatgcgatgtttcgcttggtggtcgaatgggcaggtagccggatcaagcgtatgcagccgccgcattgcatcagccatgatggatactttctcggcaggagcaaggtgagatgacaggagatcctgccccggcacttcgcccaatagcagccagtcccttcccgcttcagtgacaacgtcgagcacagctgcgcaaggaacgcccgtcgtggccagccacgatagccgcgctgcctcgtcctgcagttcattcagggcaccggacaggtcggtcttgacaaaaagaaccgggcgcccctgcgctgacagccggaacacggcggcatcagagcagccgattgtctgttgtgcccagtcatagccgaatagcctctccacccaagcggccggagaacctgcgtgcaatccatcttgttcaatggccgatcccatggtttagttcctcaccttgtcgtattatactatgccgatatactatgccgatgattaattgtcaacacgtctaacaaaaaagccaaaaacggccagaatttagcggacaatttactagtctaacactgaaaattacatattgacccaaatgattacatttcaaaaggtgcctaaaaaacttcacaaaacacactcgccaaccccgagcgcatagttcaaaaccggagcttcagctacttaagaagataggtacataaaaccgaccaaagaaactgacgcctcacttatccctcccctcaccagaggtccggcgcctgtcgattcaggagagcctaccctaggcccgaaccctgcgtcctgcgacggagaaaagcctaccgcacacctaccggcaggtggccccaccctgcattataagccaacagaacgggtgacgtcacgacacgacgagggcgcgcgctcccaaaggtacgggtgcactgcccaacggcaccgccataactgccgcccccgcaacagacgacaaaccgagttctccagtcagtgacaaacttcacgtcagggtccccagatggtgccccagcccatctcacccgaataagagctttcccgcattagcgaaggcctcaagaccttgggttcttgccgcccaccatgccccccaccttgtttcaacgacctcacagcccgcctcacaagcgtcttccattcaagactcgggaacagccgccattttgctgcgctccccccaacccccagttcagggcaaccttgctcgcggacccagactacagcccttggcggtctctccacacgcttccgtcccaccgagcggcccggcggccacgaaagccccggccagcccagcagcccgctactcaccaagtgacgatcacagcgatccacaaacaagaaccgcgacccaaatcccggctgcgacggaactagctgtgccacacccggcgcgtccttatataatcatcggcgttcaccgccccacggagatccctccgcagaatcgccgagaagggactacttttcctcgcctgttccgctctctggaaagaaaaccagtgccctagagtcacccaagtcccgtcctaaaatgtccttctgctgatactggggttctaaggccgagtcttatgagcagcgggccgctgtcctgagcgtccgggcggaaggatcaggacgctcgctgcgcccttcgtctgacgtggcagcgctcgccgtgaggaggggggcgcccgcgggaggcgccaaaacccggcgcggaggccatgcatataacttcgtatagcatacattatacgaagttatctcgagcttggtaaaggaatggagaattaaggctctagatcattagtggttacactatagtattagaagtaaaaaaaagattataccaacaaaataagaacatgttaatgtacttgtaatgaataaacatgaataaagctcttatgctatataggtgcactaaacaatctactagaattgtcagcaaactacgtatcttaatcctgaaagggtcccaaaccaatgatctaaaattgaatcaaactttcttccttgagcataattacttaaatgatttattaaaatagccagcatttaaaagcttaaaatgtaaatatcataatgtggtatcctagatagcatcccagaacagaaaaaggatattagggaaaaactggaggaatggaataaattatgcagtttagttattaataatgtactaacgtccttagttatgacgattgtaccatggtaatgtaagatactaacaatagaggaaaccgggtaaggagtatacagtaactctatactatctttgcaacttttttgtaaatttaaaacttctaaaataaagaacaaatttaaacattaaaaagtatcaccaggaacatatatcactgtttacagatgaaatactatgtattttcatatctaatttctgatcattgacttcaaatcagaaaagtgaatgacacctcaaaatcaggttttctgtttactgaagtctaagaaaagaaagcataccagctggagagattcatgtttataaagacagatttataacaacaaaaataaaatatccaagaataaatttaagaagaagcactttactgagaaacatatgaaaacctgaacaaatggagagggatattttgtatttgaatagaaagacttctggtttaaagataattctctttaaattattttttgtagaaatttaaggggtacaagagcagtgttgtcacatggatatattacatagtggtgaagtctggggttttagtgtaaattaatctttacattttgtttgagcccaataaatgtaccaacatgatttttatagaaagatagtcattcctattaatccaaacttgtcccaactttgaattgaattgaggcagagctagcaggtgttccccacggctgaggcatctgaacattaagcatatccctctgagaaccagcctgcattgatactctttctaatgtggacagcatcaagctatgtacgtagttctgtgctcagcaaaagccctgacttctttttgtttatgtcctagccccatacaacaaaatcaaccaaagaattttggttgtggatccagtcacctctgaacatgaactgacatgtcaggctgagggctaccccaaggccgaagtcatctggacaagcagtgaccatcaagtcctgagtggtaagaccaccaccaccaattccaagagagaggagaagcttttcaatgtgaccagcacactgagaatcaacacaacaactaatgagattttctactgcacttttaggagattagatcctgaggaaaaccatacagctgaattggtcatcccaggtaatattctgaatgtgtccattaaaatatgtctaacactgtcccctagcacctagcatgatgtctgcctatcatagtcattcagtgattgttgaataaatgaatgaatgaataacactatgtttacaaaatatatcctaattcctcacctccattcatccaaaccatattgttacttaataaacattcagcagatatttatggaatataccttttgttccatgcattgtagtactcattggatacacatagaataataagactcagttcacactcttcaggaaacagataaaaaactaagaaacaaacaaaaaacaggcaatccaacaccatgtgggaaatgctttcatagccgggaaacctggggaatacctgagaggaatactcaattcaggccttgtttcaggaatccaaatcctggcacatcagagctgcttccctctttccagggtggcaggaaataaatggaacatatttttctatcttatgccaaacatgagggaccctttctccccggtgcctctcccaaggtagtctacaatatttcaactctagcagtctgcttagtgcatagaacatgaggctgtgtgtccctgggcaaattactagacttctgtgtgcttcactttccctgtaggattataatctactgagcaagcttattgtaagggtcagattagcaacagtgtatgaaaatgatttgagaccattgcctgcacaaattcaactatttttttttatctcactactctacagaagtaggtagggtgggagacagagtctgatgagaggctcagaatgtgaaagaaagtgaggcgagtgagcatgatatttaatataaacacaaagatattctgagaagagctgctcactgccccctcccccaatacatgttgataggaaaatgccacgtacttcagcaaaaacaactgaaaaattagatagaaaagtcaatcaataggaaaagataatccaggacggtgttgtgaacagaaagagggggaaaaaactttagaaaatgatggggatgctcttactggggtacgagtcctcaggtattgaactggctttcagtaaaagctagattagtgggttcctgccatttacaagctgttttatgacaacttacttgttgggtggcctacagtaactcacctaactgcactgagtctgtttcctcatctgtaaattggggatttttttttaaatacctggcatgcctaactcataaagttgttctgaaactgaaataaaacatacgtgaacaggcattgtaaactgtaagttacggaaaaagctggctgttgttgtgtctttaaagtttcacctgggtagtcaaagatggatcatgggtctcagtggagagctgagccaggcaggagctgactaagggtgagaggtgggagttagcagcctctgaacatctgtgtaccatgggaccccctttcctcctgcatggtaccccagacaaggagcctagtaagagatactaatggcttgttgtccagagatgttcaaactgcagagaaagataagacaacaagcattggcctccaatcatgatgacagataggaggaggtgggagctccttagcagtgctggttggccttccatgttctactgtgggccatctctgccatgtactgtaggctactagcttctatattaaagaatgcaagaggggccaggagcggaggctcatgcctgtaatctcagcactttgggaggccaaggtgggcagatcacttgaggtcaggagtttgtgaccagcctggccaacatggtgaaactctgcctttactaaaaatataaaaattagctgggtgtggtggtgtgcacctgtaatcccagctactcgggagactgaggcacaagaattgcttgaacctgggaggcggaagttgcagtgagcccagattgcgccactgcactccaccctgggcaacagagaaagactctgcctcaaaaaaaaaaaaaaaaagcaagaggaagtgaaataatcaaggccgccatttaatagtgagcagccactccatgtggtactgtgcaagcacattataaatattagcctcacaagaaatgtattagcatttgtattttgtacactggttaagtatcttgcccaagacctcaaaactggttaagggcagcagaatttagccccagcaccaccttttcaaagcctgggcttctcacacttctccatgctgttcccattttaacacaggtatctcgccattccagccactcaaactttggcatttaagaaaattatcctaaagctaaactaaacttcaaggatgaccattctcctgaccccttcccatcaaaattttatctttagtcagtttgttttcgttttgttttgtttttcagaactacctctggcacatcctccaaatgaaagg

SEQ ID NO: 8 - DNA, 8521 bp, Artificial Sequence
  Polynucleotide (humanization fragment B)
gtcacggttcccaaggacctatatgtggtagagtatggtagcaatatgacaattgaatgcaaattcccagtagaaaaacaattagacctggctgcactaattgtctattgggaaatggaggataagaacattattcaatttgtgcatggagaggaagacctgaaggttcagcatagtagctacagacagagggcccggctgttgaaggaccagctctccctgggaaatgctgcacttcagatcacagatgtgaaattgcaggatgcaggggtgtaccgctgcatgatcagctatggtggtgccgactacaagcgaattactgtgaaagtcaatggtaagaattattatagatgagaggcctgatctttattgaaaacatattccaagtgttgaagacttttcattcttgtaagtccatacttattttcaaacagaacagcatagtctgttcattcattcattcaattcatgaattcattcacataattatccaatttcttgagcacctatttgatagtcactggaaatccagagacaaacaacacagagccatgttctacagtatgtacagttttccaaaaagaatttctagtctttacttttttattacaaatggaatacgtatacttgcaaataattcagatactgtggaagagatcaaatgaattgcaaaagtgtccctcctcccttcaccactatctcccatggcatgcagagagagtaaccattatttgtgtgtccctccagaaatttttttattcaactactatttttttattttattaggtccgtcagttttccttttttgagcctctctatatcaaatgcaaataaatatattcagaacaaaccccactgtaaggttcacattaaaaaagacttgaagtcaccctatgaagacaaaaaataatcacattaagtgtgaaagaacctattcttccagtacaggataagccatacttactgggcatatattcatcttgaaaatctatactgatgttgtcttggggaattgaaaaggaactaggagtgttagttcctcggtattgacccacagttatgttatcaggtcacttgagttcaaagttttgtgttggcactagctaagtaaaggaaaacacctctgctttcattgttgagtttcacagaattgagagctgaaaggatcccaggcaggagcagctaatccaaactcccacaaagaacaaaaatcccccagaggatcttctgttcttatatttcctgcaatggcgtccctgtcatatcccacaatggcctccctgccatttggatatcccttccatatcctgttgaaattactccctaatagtaagctgaaatctgcccctctagttgtagtcttgggattatttcatttacatgatgaccttttaatatttgactagaattaaatcatctccccttggtctttccattcctgggctaactaccatcaatctgagggctaacaatacaagtagaaaaagtatacatttgtcactgatcactgatcaattattaatcaatgatcactgataactataaactcaaaaacaaaatcatgtggggattaagagaaatgtatcagttttatgttgtatttctggtccctgatactggctcaggtaatgccactattgtcaagaagataccacttgtaaagtagatttaattttcattatattttaccatatgcttctccattcatgacatctcttgagatgttgtggtttatactttcagtttttctccagtccatccgcaaatatcaggcatctactgtgttccaagatattaaagaaatcatcatgacttagcctcatcaacagcattgctagatctgggatggaaaggaagagtataatcctggcagtcaggaagaaggcagcataaagtataagtttctgcttccaaaaaaggtctctcatcagcctgtagggagtgtgtagggaagggacagctgtccttgtagtagggaagggttttattcaggtcgtctgggctccataatatcccttgtgtatctgcagtctcctttgccatggatcaacacaataggaaatcttccggcactgatggtttttccaagggggagttcttcctggagcaaagcaaatgaccaaccaggtttgaggacctgatttgtttgacaattccattttgtattgtaaattacttaattggcattctactcccaatccatcttgtcatttgcatacagtggttttgggattgagttcagctataccaaaagtctgaaccttctgcacttagaacaaggcaaccaccaagcttcacttgcactgaggccgtgtctccaatggaaatgaggcagctggcttgcaggagcttcccaactcagggaagtagaactcctgagtcacctccatatgcaaatgatttcacagtaatgctgttgaacttcacttcccatcacagcaaatgtgtggtaacatagcttccccacaggagtttactcaccatggtattttaaaggtgaaacatttcaaaactgaaatttgaaagaatttagttttggattcactcaattatcactatcacttcgggtgttattgcacctttcttgtttgtgagtttaaatgccagactctcaggccactaactttcaattaaaagtgtttttctttaatcgctgaacctaacagcagggaaaacgaaatgttcattcagactttcagaaccttcaatgagattaggcagctgaaagatcaaagtgttgcatagttgtcccgataaagctatttggatcatatggaccaaatcgactgctgtcattccccaccaaccccatctctccccaaaattcccagccctgtttaagtgttctctgtagcatttatctctatctagtatattgtgtagcatatcatatcatacttttctgttttgtttattgtctctctcctcctagaatataaactccacaagcacaaagatttgggcctgttttataatattgttgcatccccagggcctgatatacagcagagtggtggtacgaaaagagcacacaaaaaaatatttgttgagtcaatgaatgaatgatttcctcaaataggattagcctaaaattttggaaacatgaacagatttggatatgtgaaaatttatttccagactgttcatcaggaactgttagcagcttctaaagggtacactggagcagcagtagtaaaaggaggaagaggagcagctctgctactgctactatcgagtactactacaattagcacttgcttattctgtgtgttaggccctgtactgaacactctgtctaaattagttcatttcctcctggaaatgactctagggggtaagtgcttcatcatgtaagatgagtatttttcacattttgttgtgtctgaaatctgagtgtgtctttcaatgatggaatctttgattccatgataagtggtattattcccattttaaggatgaggaaactgaggtccaaagaaattaagtaatttgcccaaattcacccagcctagaaaatgataaagctagttctaaacccaagcagattagctctgaagtctgggcccttaataaccactttttattgcctatatttgtacctctggtgtacgtatcaagttatatgttgacttcaaaactatcatgaccttttcttggttttgattgtccaacattagtatagtgttctgggtctgcaaaaattttgattactcatctcatctgtaaaacattttgaactcgtgtgtttgtgcatgcacatttgtgtgtaattataaaaattttactttctgttaatatataagttgtatcataagaaactgccgtttttgaagagcaaaaaaaggttgaatgttaccagttacatctggttcaacctaatagacatttgtacaaaaacagacattttaagaggttgaaataaaaatttaataaacaatattttcagtttttactaattgtgatgcttcactatcattagctaatatgtcaaggcataatataccttagggtgaactttatcattaacaaaggtggatggtgtcaataatcttgaggtttgtgtttttttatataacactgcgaggtctaattaagtacttactgtttaccacctcatacagtggccgataaaaagtgtcacttctgctgtttcctctgggttgtgcttgaattattagtattatcttcagtcctcagtttctttgtgggaaactttttaattagttgtttaattttgtaagatggttagtttagtcaaaattagataagagaatttgaaaatccgtagctaccccaaagcaacctacacataagaactattatttttgtgttttgaaatcataattttattgatttccagtgtttccactggtagtggtttcattgatataggagtatcaaaacatcactcattatttatttcagtttcatttgatcctagccgttttgtattaactctctgtgaagaaattacctcacaaatctattgctgtcgctagctcgctaccttaggaccgttatagttactagcataacttcgtatagcatacattatacgaagttatctcgagcttggtaaaggaatggagaattaaggctctagatcattagtggttacactatagtattagaagtaaaaaaaagattataccaacaaaataagaacatgttaatgtacttgtaatgaataaacatgaataaagctcttatgctatataggtgcactaaacaatctactagaattgtcagcaaactacgtatcttaatcctgaaagggtcccaaaccaatgatctaaaattgaatcaaactttcttccttgagcataattacttaaatgatttattaaaatagccagcatttaaaagcttaaaatgtaaatatcataatgtggtatcctagatagcatcccagaacagaaaaaggatattagggaaaaactggaggaatggaataaattatgcagtttagttattaataatgtactaacgtccttagttatgacgattgtaccatggtaatgtaagatactaacaatagaggaaaccgggtaaggagtatacagtaactctatactatctttgcaacttttttgtaaatttaaaacttctaaaataaagaacaaatttaaacattaaaaagtatcaccaggaacatatatcactgtttacagatgaaatactatgtattttcatatctaatttctgatcattgacttcaaatcagaaaagtgaatgacacctcaaaatcaggttttctgtttactgaagtctaagaaaagaaagcataccagctggagagattcatgtttataaagacagatttataacaacaaaaataaaatatccaagaataaatttaagaagaagcactttactgagaaacatatgaaaacctgaacaaatggagagggatattttgtatttgaatagaaagacttctggtttaaagataattctctttaaattattttttgtagaaatttaaggggtacaagagcagtgttgtcacatggatatattacatagtggtgaagtctggggttttagtgtaaattaatctttacattttgtttgagcccaataaatgtaccaacatgatttttatagaaagatagtcattcctattaatccaaacttgtcccaactttgaattgaattgaggcagagctagcaggtgttccccacggctgaggcatctgaacattaagcatatccctctgagaaccagcctgcattgatactctttctaatgtggacagcatcaagctatgtacgtagttctgtgctcagcaaaagccctgacttctttttgtttatgtcctagccccatacaacaaaatcaaccaaagaattttggttgtggatccagtcacctctgaacatgaactgacatgtcaggctgagggctaccccaaggccgaagtcatctggacaagcagtgaccatcaagtcctgagtggtaagaccaccaccaccaattccaagagagaggagaagcttttcaatgtgaccagcacactgagaatcaacacaacaactaatgagattttctactgcacttttaggagattagatcctgaggaaaaccatacagctgaattggtcatcccaggtaatattctgaatgtgtccattaaaatatgtctaacactgtcccctagcacctagcatgatgtctgcctatcatagtcattcagtgattgttgaataaatgaatgaatgaataacactatgtttacaaaatatatcctaattcctcacctccattcatccaaaccatattgttacttaataaacattcagcagatatttatggaatataccttttgttccatgcattgtagtactcattggatacacatagaataataagactcagttcacactcttcaggaaacagataaaaaactaagaaacaaacaaaaaacaggcaatccaacaccatgtgggaaatgctttcatagccgggaaacctggggaatacctgagaggaatactcaattcaggccttgtttcaggaatccaaatcctggcacatcagagctgcttccctctttccagggtggcaggaaataaatggaacatatttttctatcttatgccaaacatgagggaccctttctccccggtgcctctcccaaggtagtctacaatatttcaactctagcagtctgcttagtgcatagaacatgaggctgtgtgtccctgggcaaattactagacttctgtgtgcttcactttccctgtaggattataatctactgagcaagcttattgtaagggtcagattagcaacagtgtatgaaaatgatttgagaccattgcctgcacaaattcaactatttttttttatctcactactctacagaagtaggtagggtgggagacagagtctgatgagaggctcagaatgtgaaagaaagtgaggcgagtgagcatgatatttaatataaacacaaagatattctgagaagagctgctcactgccccctcccccaatacatgttgataggaaaatgccacgtacttcagcaaaaacaactgaaaaattagatagaaaagtcaatcaataggaaaagataatccaggacggtgttgtgaacagaaagagggggaaaaaactttagaaaatgatggggatgctcttactggggtacgagtcctcaggtattgaactggctttcagtaaaagctagattagtgggttcctgccatttacaagctgttttatgacaacttacttgttgggtggcctacagtaactcacctaactgcactgagtctgtttcctcatctgtaaattggggatttttttttaaatacctggcatgcctaactcataaagttgttctgaaactgaaataaaacatacgtgaacaggcattgtaaactgtaagttacggaaaaagctggctgttgttgtgtctttaaagtttcacctgggtagtcaaagatggatcatgggtctcagtggagagctgagccaggcaggagctgactaagggtgagaggtgggagttagcagcctctgaacatctgtgtaccatgggaccccctttcctcctgcatggtaccccagacaaggagcctagtaagagatactaatggcttgttgtccagagatgttcaaactgcagagaaagataagacaacaagcattggcctccaatcatgatgacagataggaggaggtgggagctccttagcagtgctggttggccttccatgttctactgtgggccatctctgccatgtactgtaggctactagcttctatattaaagaatgcaagaggggccaggagcggaggctcatgcctgtaatctcagcactttgggaggccaaggtgggcagatcacttgaggtcaggagtttgtgaccagcctggccaacatggtgaaactctgcctttactaaaaatataaaaattagctgggtgtggtggtgtgcacctgtaatcccagctactcgggagactgaggcacaagaattgcttgaacctgggaggcggaagttgcagtgagcccagattgcgccactgcactccaccctgggcaacagagaaagactctgcctcaaaaaaaaaaaaaaaaagcaagaggaagtgaaataatcaaggccgccatttaatagtgagcagccactccatgtggtactgtgcaagcacattataaatattagcctcacaagaaatgtattagcatttgtattttgtacactggttaagtatcttgcccaagacctcaaaactggttaagggcagcagaatttagccccagcaccaccttttcaaagcctgggcttctcacacttctccatgctgttcccattttaacacaggtatctcgccattccagccactcaaactttggcatttaagaaaattatcctaaagctaaactaaacttcaaggatgaccattctcctgaccccttcccatcaaaattttatctttagtcagtttgttttcgttttgttttgtttttcagaactacctctggcacatcctccaaatgaaagg

SEQ ID NO: 9 - DNA, 4494 bp, Artificial Sequence
  Polynucleotide (humanization fragment C)
gtcacggttcccaaggacctatatgtggtagagtatggtagcaatatgacaattgaatgcaaattcccagtagaaaaacaattagacctggctgcactaattgtctattgggaaatggaggataagaacattattcaatttgtgcatggagaggaagacctgaaggttcagcatagtagctacagacagagggcccggctgttgaaggaccagctctccctgggaaatgctgcacttcagatcacagatgtgaaattgcaggatgcaggggtgtaccgctgcatgatcagctatggtggtgccgactacaagcgaattactgtgaaagtcaatggtaagaattattatagatgagaggcctgatctttattgaaaacatattccaagtgttgaagacttttcattcttgtaagtccatacttattttcaaacagaacagcatagtctgttcattcattcattcaattcatgaattcattcacataattatccaatttcttgagcacctatttgatagtcactggaaatccagagacaaacaacacagagccatgttctacagtatgtacagttttccaaaaagaatttctagtctttacttttttattacaaatggaatacgtatacttgcaaataattcagatactgtggaagagatcaaatgaattgcaaaagtgtccctcctcccttcaccactatctcccatggcatgcagagagagtaaccattatttgtgtgtccctccagaaatttttttattcaactactatttttttattttattaggtccgtcagttttccttttttgagcctctctatatcaaatgcaaataaatatattcagaacaaaccccactgtaaggttcacattaaaaaagacttgaagtcaccctatgaagacaaaaaataatcacattaagtgtgaaagaacctattcttccagtacaggataagccatacttactgggcatatattcatcttgaaaatctatactgatgttgtcttggggaattgaaaaggaactaggagtgttagttcctcggtattgacccacagttatgttatcaggtcacttgagttcaaagttttgtgttggcactagctaagtaaaggaaaacacctctgctttcattgttgagtttcacagaattgagagctgaaaggatcccaggcaggagcagctaatccaaactcccacaaagaacaaaaatcccccagaggatcttctgttcttatatttcctgcaatggcgtccctgtcatatcccacaatggcctccctgccatttggatatcccttccatatcctgttgaaattactccctaatagtaagctgaaatctgcccctctagttgtagtcttgggattatttcatttacatgatgaccttttaatatttgactagaattaaatcatctccccttggtctttccattcctgggctaactaccatcaatctgagggctaacaatacaagtagaaaaagtatacatttgtcactgatcactgatcaattattaatcaatgatcactgataactataaactcaaaaacaaaatcatgtggggattaagagaaatgtatcagttttatgttgtatttctggtccctgatactggctcaggtaatgccactattgtcaagaagataccacttgtaaagtagatttaattttcattatattttaccatatgcttctccattcatgacatctcttgagatgttgtggtttatactttcagtttttctccagtccatccgcaaatatcaggcatctactgtgttccaagatattaaagaaatcatcatgacttagcctcatcaacagcattgctagatctgggatggaaaggaagagtataatcctggcagtcaggaagaaggcagcataaagtataagtttctgcttccaaaaaaggtctctcatcagcctgtagggagtgtgtagggaagggacagctgtccttgtagtagggaagggttttattcaggtcgtctgggctccataatatcccttgtgtatctgcagtctcctttgccatggatcaacacaataggaaatcttccggcactgatggtttttccaagggggagttcttcctggagcaaagcaaatgaccaaccaggtttgaggacctgatttgtttgacaattccattttgtattgtaaattacttaattggcattctactcccaatccatcttgtcatttgcatacagtggttttgggattgagttcagctataccaaaagtctgaaccttctgcacttagaacaaggcaaccaccaagcttcacttgcactgaggccgtgtctccaatggaaatgaggcagctggcttgcaggagcttcccaactcagggaagtagaactcctgagtcacctccatatgcaaatgatttcacagtaatgctgttgaacttcacttcccatcacagcaaatgtgtggtaacatagcttccccacaggagtttactcaccatggtattttaaaggtgaaacatttcaaaactgaaatttgaaagaatttagttttggattcactcaattatcactatcacttcgggtgttattgcacctttcttgtttgtgagtttaaatgccagactctcaggccactaactttcaattaaaagtgtttttctttaatcgctgaacctaacagcagggaaaacgaaatgttcattcagactttcagaaccttcaatgagattaggcagctgaaagatcaaagtgttgcatagttgtcccgataaagctatttggatcatatggaccaaatcgactgctgtcattccccaccaaccccatctctccccaaaattcccagccctgtttaagtgttctctgtagcatttatctctatctagtatattgtgtagcatatcatatcatacttttctgttttgtttattgtctctctcctcctagaatataaactccacaagcacaaagatttgggcctgttttataatattgttgcatccccagggcctgatatacagcagagtggtggtacgaaaagagcacacaaaaaaatatttgttgagtcaatgaatgaatgatttcctcaaataggattagcctaaaattttggaaacatgaacagatttggatatgtgaaaatttatttccagactgttcatcaggaactgttagcagcttctaaagggtacactggagcagcagtagtaaaaggaggaagaggagcagctctgctactgctactatcgagtactactacaattagcacttgcttattctgtgtgttaggccctgtactgaacactctgtctaaattagttcatttcctcctggaaatgactctagggggtaagtgcttcatcatgtaagatgagtatttttcacattttgttgtgtctgaaatctgagtgtgtctttcaatgatggaatctttgattccatgataagtggtattattcccattttaaggatgaggaaactgaggtccaaagaaattaagtaatttgcccaaattcacccagcctagaaaatgataaagctagttctaaacccaagcagattagctctgaagtctgggcccttaataaccactttttattgcctatatttgtacctctggtgtacgtatcaagttatatgttgacttcaaaactatcatgaccttttcttggttttgattgtccaacattagtatagtgttctgggtctgcaaaaattttgattactcatctcatctgtaaaacattttgaactcgtgtgtttgtgcatgcacatttgtgtgtaattataaaaattttactttctgttaatatataagttgtatcataagaaactgccgtttttgaagagcaaaaaaaggttgaatgttaccagttacatctggttcaacctaatagacatttgtacaaaaacagacattttaagaggttgaaataaaaatttaataaacaatattttcagtttttactaattgtgatgcttcactatcattagctaatatgtcaaggcataatataccttagggtgaactttatcattaacaaaggtggatggtgtcaataatcttgaggtttgtgtttttttatataacactgcgaggtctaattaagtacttactgtttaccacctcatacagtggccgataaaaagtgtcacttctgctgtttcctctgggttgtgcttgaattattagtattatcttcagtcctcagtttctttgtgggaaactttttaattagttgtttaattttgtaagatggttagtttagtcaaaattagataagagaatttgaaaatccgtagctaccccaaagcaacctacacataagaactattatttttgtgttttgaaatcataattttattgatttccagtgtttccactggtagtggtttcattgatataggagtatcaaaacatcactcattatttatttcagtttcatttgatcctagccgttttgtattaactctctgtgaagaaattacctcacaaatctattgctgtc

SEQ ID NO: 10 - DNA, 3950 bp, Artificial Sequence
  Polynucleotide (humanization fragment D)
cttggtaaaggaatggagaattaaggctctagatcattagtggttacactatagtattagaagtaaaaaaaagattataccaacaaaataagaacatgttaatgtacttgtaatgaataaacatgaataaagctcttatgctatataggtgcactaaacaatctactagaattgtcagcaaactacgtatcttaatcctgaaagggtcccaaaccaatgatctaaaattgaatcaaactttcttccttgagcataattacttaaatgatttattaaaatagccagcatttaaaagcttaaaatgtaaatatcataatgtggtatcctagatagcatcccagaacagaaaaaggatattagggaaaaactggaggaatggaataaattatgcagtttagttattaataatgtactaacgtccttagttatgacgattgtaccatggtaatgtaagatactaacaatagaggaaaccgggtaaggagtatacagtaactctatactatctttgcaacttttttgtaaatttaaaacttctaaaataaagaacaaatttaaacattaaaaagtatcaccaggaacatatatcactgtttacagatgaaatactatgtattttcatatctaatttctgatcattgacttcaaatcagaaaagtgaatgacacctcaaaatcaggttttctgtttactgaagtctaagaaaagaaagcataccagctggagagattcatgtttataaagacagatttataacaacaaaaataaaatatccaagaataaatttaagaagaagcactttactgagaaacatatgaaaacctgaacaaatggagagggatattttgtatttgaatagaaagacttctggtttaaagataattctctttaaattattttttgtagaaatttaaggggtacaagagcagtgttgtcacatggatatattacatagtggtgaagtctggggttttagtgtaaattaatctttacattttgtttgagcccaataaatgtaccaacatgatttttatagaaagatagtcattcctattaatccaaacttgtcccaactttgaattgaattgaggcagagctagcaggtgttccccacggctgaggcatctgaacattaagcatatccctctgagaaccagcctgcattgatactctttctaatgtggacagcatcaagctatgtacgtagttctgtgctcagcaaaagccctgacttctttttgtttatgtcctagccccatacaacaaaatcaaccaaagaattttggttgtggatccagtcacctctgaacatgaactgacatgtcaggctgagggctaccccaaggccgaagtcatctggacaagcagtgaccatcaagtcctgagtggtaagaccaccaccaccaattccaagagagaggagaagcttttcaatgtgaccagcacactgagaatcaacacaacaactaatgagattttctactgcacttttaggagattagatcctgaggaaaaccatacagctgaattggtcatcccaggtaatattctgaatgtgtccattaaaatatgtctaacactgtcccctagcacctagcatgatgtctgcctatcatagtcattcagtgattgttgaataaatgaatgaatgaataacactatgtttacaaaatatatcctaattcctcacctccattcatccaaaccatattgttacttaataaacattcagcagatatttatggaatataccttttgttccatgcattgtagtactcattggatacacatagaataataagactcagttcacactcttcaggaaacagataaaaaactaagaaacaaacaaaaaacaggcaatccaacaccatgtgggaaatgctttcatagccgggaaacctggggaatacctgagaggaatactcaattcaggccttgtttcaggaatccaaatcctggcacatcagagctgcttccctctttccagggtggcaggaaataaatggaacatatttttctatcttatgccaaacatgagggaccctttctccccggtgcctctcccaaggtagtctacaatatttcaactctagcagtctgcttagtgcatagaacatgaggctgtgtgtccctgggcaaattactagacttctgtgtgcttcactttccctgtaggattataatctactgagcaagcttattgtaagggtcagattagcaacagtgtatgaaaatgatttgagaccattgcctgcacaaattcaactatttttttttatctcactactctacagaagtaggtagggtgggagacagagtctgatgagaggctcagaatgtgaaagaaagtgaggcgagtgagcatgatatttaatataaacacaaagatattctgagaagagctgctcactgccccctcccccaatacatgttgataggaaaatgccacgtacttcagcaaaaacaactgaaaaattagatagaaaagtcaatcaataggaaaagataatccaggacggtgttgtgaacagaaagagggggaaaaaactttagaaaatgatggggatgctcttactggggtacgagtcctcaggtattgaactggctttcagtaaaagctagattagtgggttcctgccatttacaagctgttttatgacaacttacttgttgggtggcctacagtaactcacctaactgcactgagtctgtttcctcatctgtaaattggggatttttttttaaatacctggcatgcctaactcataaagttgttctgaaactgaaataaaacatacgtgaacaggcattgtaaactgtaagttacggaaaaagctggctgttgttgtgtctttaaagtttcacctgggtagtcaaagatggatcatgggtctcagtggagagctgagccaggcaggagctgactaagggtgagaggtgggagttagcagcctctgaacatctgtgtaccatgggaccccctttcctcctgcatggtaccccagacaaggagcctagtaagagatactaatggcttgttgtccagagatgttcaaactgcagagaaagataagacaacaagcattggcctccaatcatgatgacagataggaggaggtgggagctccttagcagtgctggttggccttccatgttctactgtgggccatctctgccatgtactgtaggctactagcttctatattaaagaatgcaagaggggccaggagcggaggctcatgcctgtaatctcagcactttgggaggccaaggtgggcagatcacttgaggtcaggagtttgtgaccagcctggccaacatggtgaaactctgcctttactaaaaatataaaaattagctgggtgtggtggtgtgcacctgtaatcccagctactcgggagactgaggcacaagaattgcttgaacctgggaggcggaagttgcagtgagcccagattgcgccactgcactccaccctgggcaacagagaaagactctgcctcaaaaaaaaaaaaaaaaagcaagaggaagtgaaataatcaaggccgccatttaatagtgagcagccactccatgtggtactgtgcaagcacattataaatattagcctcacaagaaatgtattagcatttgtattttgtacactggttaagtatcttgcccaagacctcaaaactggttaagggcagcagaatttagccccagcaccaccttttcaaagcctgggcttctcacacttctccatgctgttcccattttaacacaggtatctcgccattccagccactcaaactttggcatttaagaaaattatcctaaagctaaactaaacttcaaggatgaccattctcctgaccccttcccatcaaaattttatctttagtcagtttgttttcgttttgttttgtttttcagaactacctctggcacatcctccaaatgaaagg

SEQ ID NO: 11 - DNA, 8444 bp, Artificial Sequence
  Polynucleotide (humanization fragment E)
gtcacggttcccaaggacctatatgtggtagagtatggtagcaatatgacaattgaatgcaaattcccagtagaaaaacaattagacctggctgcactaattgtctattgggaaatggaggataagaacattattcaatttgtgcatggagaggaagacctgaaggttcagcatagtagctacagacagagggcccggctgttgaaggaccagctctccctgggaaatgctgcacttcagatcacagatgtgaaattgcaggatgcaggggtgtaccgctgcatgatcagctatggtggtgccgactacaagcgaattactgtgaaagtcaatggtaagaattattatagatgagaggcctgatctttattgaaaacatattccaagtgttgaagacttttcattcttgtaagtccatacttattttcaaacagaacagcatagtctgttcattcattcattcaattcatgaattcattcacataattatccaatttcttgagcacctatttgatagtcactggaaatccagagacaaacaacacagagccatgttctacagtatgtacagttttccaaaaagaatttctagtctttacttttttattacaaatggaatacgtatacttgcaaataattcagatactgtggaagagatcaaatgaattgcaaaagtgtccctcctcccttcaccactatctcccatggcatgcagagagagtaaccattatttgtgtgtccctccagaaatttttttattcaactactatttttttattttattaggtccgtcagttttccttttttgagcctctctatatcaaatgcaaataaatatattcagaacaaaccccactgtaaggttcacattaaaaaagacttgaagtcaccctatgaagacaaaaaataatcacattaagtgtgaaagaacctattcttccagtacaggataagccatacttactgggcatatattcatcttgaaaatctatactgatgttgtcttggggaattgaaaaggaactaggagtgttagttcctcggtattgacccacagttatgttatcaggtcacttgagttcaaagttttgtgttggcactagctaagtaaaggaaaacacctctgctttcattgttgagtttcacagaattgagagctgaaaggatcccaggcaggagcagctaatccaaactcccacaaagaacaaaaatcccccagaggatcttctgttcttatatttcctgcaatggcgtccctgtcatatcccacaatggcctccctgccatttggatatcccttccatatcctgttgaaattactccctaatagtaagctgaaatctgcccctctagttgtagtcttgggattatttcatttacatgatgaccttttaatatttgactagaattaaatcatctccccttggtctttccattcctgggctaactaccatcaatctgagggctaacaatacaagtagaaaaagtatacatttgtcactgatcactgatcaattattaatcaatgatcactgataactataaactcaaaaacaaaatcatgtggggattaagagaaatgtatcagttttatgttgtatttctggtccctgatactggctcaggtaatgccactattgtcaagaagataccacttgtaaagtagatttaattttcattatattttaccatatgcttctccattcatgacatctcttgagatgttgtggtttatactttcagtttttctccagtccatccgcaaatatcaggcatctactgtgttccaagatattaaagaaatcatcatgacttagcctcatcaacagcattgctagatctgggatggaaaggaagagtataatcctggcagtcaggaagaaggcagcataaagtataagtttctgcttccaaaaaaggtctctcatcagcctgtagggagtgtgtagggaagggacagctgtccttgtagtagggaagggttttattcaggtcgtctgggctccataatatcccttgtgtatctgcagtctcctttgccatggatcaacacaataggaaatcttccggcactgatggtttttccaagggggagttcttcctggagcaaagcaaatgaccaaccaggtttgaggacctgatttgtttgacaattccattttgtattgtaaattacttaattggcattctactcccaatccatcttgtcatttgcatacagtggttttgggattgagttcagctataccaaaagtctgaaccttctgcacttagaacaaggcaaccaccaagcttcacttgcactgaggccgtgtctccaatggaaatgaggcagctggcttgcaggagcttcccaactcagggaagtagaactcctgagtcacctccatatgcaaatgatttcacagtaatgctgttgaacttcacttcccatcacagcaaatgtgtggtaacatagcttccccacaggagtttactcaccatggtattttaaaggtgaaacatttcaaaactgaaatttgaaagaatttagttttggattcactcaattatcactatcacttcgggtgttattgcacctttcttgtttgtgagtttaaatgccagactctcaggccactaactttcaattaaaagtgtttttctttaatcgctgaacctaacagcagggaaaacgaaatgttcattcagactttcagaaccttcaatgagattaggcagctgaaagatcaaagtgttgcatagttgtcccgataaagctatttggatcatatggaccaaatcgactgctgtcattccccaccaaccccatctctccccaaaattcccagccctgtttaagtgttctctgtagcatttatctctatctagtatattgtgtagcatatcatatcatacttttctgttttgtttattgtctctctcctcctagaatataaactccacaagcacaaagatttgggcctgttttataatattgttgcatccccagggcctgatatacagcagagtggtggtacgaaaagagcacacaaaaaaatatttgttgagtcaatgaatgaatgatttcctcaaataggattagcctaaaattttggaaacatgaacagatttggatatgtgaaaatttatttccagactgttcatcaggaactgttagcagcttctaaagggtacactggagcagcagtagtaaaaggaggaagaggagcagctctgctactgctactatcgagtactactacaattagcacttgcttattctgtgtgttaggccctgtactgaacactctgtctaaattagttcatttcctcctggaaatgactctagggggtaagtgcttcatcatgtaagatgagtatttttcacattttgttgtgtctgaaatctgagtgtgtctttcaatgatggaatctttgattccatgataagtggtattattcccattttaaggatgaggaaactgaggtccaaagaaattaagtaatttgcccaaattcacccagcctagaaaatgataaagctagttctaaacccaagcagattagctctgaagtctgggcccttaataaccactttttattgcctatatttgtacctctggtgtacgtatcaagttatatgttgacttcaaaactatcatgaccttttcttggttttgattgtccaacattagtatagtgttctgggtctgcaaaaattttgattactcatctcatctgtaaaacattttgaactcgtgtgtttgtgcatgcacatttgtgtgtaattataaaaattttactttctgttaatatataagttgtatcataagaaactgccgtttttgaagagcaaaaaaaggttgaatgttaccagttacatctggttcaacctaatagacatttgtacaaaaacagacattttaagaggttgaaataaaaatttaataaacaatattttcagtttttactaattgtgatgcttcactatcattagctaatatgtcaaggcataatataccttagggtgaactttatcattaacaaaggtggatggtgtcaataatcttgaggtttgtgtttttttatataacactgcgaggtctaattaagtacttactgtttaccacctcatacagtggccgataaaaagtgtcacttctgctgtttcctctgggttgtgcttgaattattagtattatcttcagtcctcagtttctttgtgggaaactttttaattagttgtttaattttgtaagatggttagtttagtcaaaattagataagagaatttgaaaatccgtagctaccccaaagcaacctacacataagaactattatttttgtgttttgaaatcataattttattgatttccagtgtttccactggtagtggtttcattgatataggagtatcaaaacatcactcattatttatttcagtttcatttgatcctagccgttttgtattaactctctgtgaagaaattacctcacaaatctattgctgtccttggtaaaggaatggagaattaaggctctagatcattagtggttacactatagtattagaagtaaaaaaaagattataccaacaaaataagaacatgttaatgtacttgtaatgaataaacatgaataaagctcttatgctatataggtgcactaaacaatctactagaattgtcagcaaactacgtatcttaatcctgaaagggtcccaaaccaatgatctaaaattgaatcaaactttcttccttgagcataattacttaaatgatttattaaaatagccagcatttaaaagcttaaaatgtaaatatcataatgtggtatcctagatagcatcccagaacagaaaaaggatattagggaaaaactggaggaatggaataaattatgcagtttagttattaataatgtactaacgtccttagttatgacgattgtaccatggtaatgtaagatactaacaatagaggaaaccgggtaaggagtatacagtaactctatactatctttgcaacttttttgtaaatttaaaacttctaaaataaagaacaaatttaaacattaaaaagtatcaccaggaacatatatcactgtttacagatgaaatactatgtattttcatatctaatttctgatcattgacttcaaatcagaaaagtgaatgacacctcaaaatcaggttttctgtttactgaagtctaagaaaagaaagcataccagctggagagattcatgtttataaagacagatttataacaacaaaaataaaatatccaagaataaatttaagaagaagcactttactgagaaacatatgaaaacctgaacaaatggagagggatattttgtatttgaatagaaagacttctggtttaaagataattctctttaaattattttttgtagaaatttaaggggtacaagagcagtgttgtcacatggatatattacatagtggtgaagtctggggttttagtgtaaattaatctttacattttgtttgagcccaataaatgtaccaacatgatttttatagaaagatagtcattcctattaatccaaacttgtcccaactttgaattgaattgaggcagagctagcaggtgttccccacggctgaggcatctgaacattaagcatatccctctgagaaccagcctgcattgatactctttctaatgtggacagcatcaagctatgtacgtagttctgtgctcagcaaaagccctgacttctttttgtttatgtcctagccccatacaacaaaatcaaccaaagaattttggttgtggatccagtcacctctgaacatgaactgacatgtcaggctgagggctaccccaaggccgaagtcatctggacaagcagtgaccatcaagtcctgagtggtaagaccaccaccaccaattccaagagagaggagaagcttttcaatgtgaccagcacactgagaatcaacacaacaactaatgagattttctactgcacttttaggagattagatcctgaggaaaaccatacagctgaattggtcatcccaggtaatattctgaatgtgtccattaaaatatgtctaacactgtcccctagcacctagcatgatgtctgcctatcatagtcattcagtgattgttgaataaatgaatgaatgaataacactatgtttacaaaatatatcctaattcctcacctccattcatccaaaccatattgttacttaataaacattcagcagatatttatggaatataccttttgttccatgcattgtagtactcattggatacacatagaataataagactcagttcacactcttcaggaaacagataaaaaactaagaaacaaacaaaaaacaggcaatccaacaccatgtgggaaatgctttcatagccgggaaacctggggaatacctgagaggaatactcaattcaggccttgtttcaggaatccaaatcctggcacatcagagctgcttccctctttccagggtggcaggaaataaatggaacatatttttctatcttatgccaaacatgagggaccctttctccccggtgcctctcccaaggtagtctacaatatttcaactctagcagtctgcttagtgcatagaacatgaggctgtgtgtccctgggcaaattactagacttctgtgtgcttcactttccctgtaggattataatctactgagcaagcttattgtaagggtcagattagcaacagtgtatgaaaatgatttgagaccattgcctgcacaaattcaactatttttttttatctcactactctacagaagtaggtagggtgggagacagagtctgatgagaggctcagaatgtgaaagaaagtgaggcgagtgagcatgatatttaatataaacacaaagatattctgagaagagctgctcactgccccctcccccaatacatgttgataggaaaatgccacgtacttcagcaaaaacaactgaaaaattagatagaaaagtcaatcaataggaaaagataatccaggacggtgttgtgaacagaaagagggggaaaaaactttagaaaatgatggggatgctcttactggggtacgagtcctcaggtattgaactggctttcagtaaaagctagattagtgggttcctgccatttacaagctgttttatgacaacttacttgttgggtggcctacagtaactcacctaactgcactgagtctgtttcctcatctgtaaattggggatttttttttaaatacctggcatgcctaactcataaagttgttctgaaactgaaataaaacatacgtgaacaggcattgtaaactgtaagttacggaaaaagctggctgttgttgtgtctttaaagtttcacctgggtagtcaaagatggatcatgggtctcagtggagagctgagccaggcaggagctgactaagggtgagaggtgggagttagcagcctctgaacatctgtgtaccatgggaccccctttcctcctgcatggtaccccagacaaggagcctagtaagagatactaatggcttgttgtccagagatgttcaaactgcagagaaagataagacaacaagcattggcctccaatcatgatgacagataggaggaggtgggagctccttagcagtgctggttggccttccatgttctactgtgggccatctctgccatgtactgtaggctactagcttctatattaaagaatgcaagaggggccaggagcggaggctcatgcctgtaatctcagcactttgggaggccaaggtgggcagatcacttgaggtcaggagtttgtgaccagcctggccaacatggtgaaactctgcctttactaaaaatataaaaattagctgggtgtggtggtgtgcacctgtaatcccagctactcgggagactgaggcacaagaattgcttgaacctgggaggcggaagttgcagtgagcccagattgcgccactgcactccaccctgggcaacagagaaagactctgcctcaaaaaaaaaaaaaaaaagcaagaggaagtgaaataatcaaggccgccatttaatagtgagcagccactccatgtggtactgtgcaagcacattataaatattagcctcacaagaaatgtattagcatttgtattttgtacactggttaagtatcttgcccaagacctcaaaactggttaagggcagcagaatttagccccagcaccaccttttcaaagcctgggcttctcacacttctccatgctgttcccattttaacacaggtatctcgccattccagccactcaaactttggcatttaagaaaattatcctaaagctaaactaaacttcaaggatgaccattctcctgaccccttcccatcaaaattttatctttagtcagtttgttttcgttttgttttgtttttcagaactacctctggcacatcctccaaatgaaagg

SEQ ID NO: 12 - DNA, 111 bp, Artificial Sequence
  Synthetic oligonucleotide
aactacctctggcacatcctccaaatgaaaggactcactgggtgcttctgggatccatcctgttgttcctcattgtagtgtccacggtcctcctcttcttgagaaaacaag

SEQ ID NO: 13 - DNA, 159 bp, Artificial Sequence
  Synthetic oligonucleotide
taaccttttacccaggttttcagatgtgtttggaggagttttctgtcttctgagggctggtcctctttccttttcagcgtttactgtcaggttcccaaggacctatatgtggtagagtatggtagcaatatgacaattgaatgcaaattcccagtagaa

SEQ ID NO: 14 - DNA, 240 bp, Artificial Sequence
  Synthetic oligonucleotide
tttgtattaactctctgtgaagaaattacctcacaaatctattgctgtcgctagctcgctaccttaggaccgttatagttactagcataacttcgtatagcatacattatacgaagttattccagacatgataagatacattgatgagtttggacaaaccacaactagaatgcagtgaaaaaaatgctttatttgtgaaatttgtgatgctattgctttatttgtaaccattataagctg

SEQ ID NO: 15 - DNA, 240 bp, Artificial Sequence
  Synthetic oligonucleotide
gtgaggaggggggcgcccgcgggaggcgccaaaacccggcgcggaggccatgcatataacttcgtatagcatacattatacgaagttatctcgagcttggtaaaggaatggagaattaaggctctagatcattagtggttacactatagtattagaagtaaaaaaaagattataccaacaaaataagaacatgttaatgtacttgtaatgaataaacatgaataaagctcttatgctata

SEQ ID NO: 16 - DNA, 169 bp, Artificial Sequence
  Synthetic oligonucleotide
tttatctttagtcagtttgttttcgttttgttttgtttttcagaactacctctggcacatcctccaaatgaaaggactcactgggtgcttctgggatccatcctgttgttcctcattgtagtgtccacggtcctcctcttcttgagaaaacaaggtatttcctccattg

SEQ ID NO: 17 - DNA, 230 bp, Artificial Sequence
  Synthetic oligonucleotide
tcctagccgttttgtattaactctctgtgaagaaattacctcacaaatctattgctgtcgctagctcgctaccttaggaccgttatagttactagcataacttcgtatagcatacattatacgaagttatctcgagcttggtaaaggaatggagaattaaggctctagatcattagtggttacactatagtattagaagtaaaaaaaagattataccaacaaaataagaa

SEQ ID NO: 18 - DNA, 19 bp, Artificial Sequence
  Synthetic oligonucleotide
ccggctgttgaaggaccag

SEQ ID NO: 19 - DNA, 26 bp, Artificial Sequence
  Synthetic oligonucleotide
tctccctgggaaatgctgcacttcag

SEQ ID NO: 20 - DNA, 23 bp, Artificial Sequence
  Synthetic oligonucleotide
tgcatcctgcaatttcacatctg

SEQ ID NO: 21 - DNA, 21 bp, Artificial Sequence
  Synthetic oligonucleotide
acacaggtatctcgccattcc

SEQ ID NO: 22 - DNA, 21 bp, Artificial Sequence
  Synthetic oligonucleotide
agccactcaaactttggcatt

SEQ ID NO: 23 - DNA, 25 bp, Artificial Sequence
  Synthetic oligonucleotide
ggtcatccttgaagtttagtttagc

SEQ ID NO: 24 - DNA, 18 bp, Artificial Sequence
  Synthetic oligonucleotide
caggacgcaggcgtttac

SEQ ID NO: 25 - DNA, 26 bp, Artificial Sequence
  Synthetic oligonucleotide
ctgcataatcagctacggtggtgcgg

SEQ ID NO: 26 - DNA, 21 bp, Artificial Sequence
  Synthetic oligonucleotide
ttcagcgtgattcgcttgtag

SEQ ID NO: 27 - DNA, 18 bp, Artificial Sequence
  Synthetic oligonucleotide
ctggagtgcccaagagtc

SEQ ID NO: 28 - DNA, 27 bp, Artificial Sequence
  Synthetic oligonucleotide
cagacatggaagaaacacaacccgcac

SEQ ID NO: 29 - DNA, 19 bp, Artificial Sequence
  Synthetic oligonucleotide
ctgctaagccgcttctgtc

SEQ ID NO: 30 - DNA, 22 bp, Artificial Sequence
  Synthetic oligonucleotide
gctctggctggtcttcagtatg

SEQ ID NO: 31 - DNA, 17 bp, Artificial Sequence
  Synthetic oligonucleotide
agcagctctgccctcat

SEQ ID NO: 32 - DNA, 22 bp, Artificial Sequence
  Synthetic oligonucleotide
ttgccgtatggttggtttgaac

SEQ ID NO: 33 - DNA, 19 bp, Artificial Sequence
  Synthetic oligonucleotide
acagcctgctgtcacttgc

SEQ ID NO: 34 - DNA, 19 bp, Artificial Sequence
  Synthetic oligonucleotide
tacgggcgtttactgtcac

SEQ ID NO: 35 - DNA, 23 bp, Artificial Sequence
  Synthetic oligonucleotide
accacatataggtccttgggaac

SEQ ID NO: 36 - DNA, 21 bp, Artificial Sequence
  Synthetic oligonucleotide
ttctcaatgtgaccagcagtc

SEQ ID NO: 37 - DNA, 23 bp, Artificial Sequence
  Synthetic oligonucleotide
agggtcaacgccacagcgaatga

SEQ ID NO: 38 - DNA, 21 bp, Artificial Sequence
  Synthetic oligonucleotide
tcctgttctgtggaggatgtg